European Patent Application EP 4 112 743 A1, published January 4, 2023. Title: Method for detecting single-stranded RNA virus. Applicant: EIKEN KAGAKU KABUSHIKI KAISHA. The sequence listing filed with the application follows.

SEQUENCE LISTING (62 sequences)

SEQ ID NO: 1 - RNA, 411 nt, Artificial sequence
  modified sequence of DENV3 capsid
guaauacgacucacuauagggaguuguuagucuacguggaccgacaagaacaguuucgacucggaagcuugcuuaacguagugcugacaguuuuuuauuagagagcagaucucugaugaacaaccaacggaaaaagacgggaaaaccgucuaucaauaugcugaaacgcgugagaaaccgugugucaacuggaucacaguuggcgaagagauucucaaaaggauugcugaacggccaaggaccaaugaaauugguuauggcguucauagcuuuccucagauuucuagccauuccaccaacagcaggagucuuggcuagauggggaaccuucaagaagucgggggccauuaagguccugaaaggcuucaagaaggagaucucaaacaugcugagcauuaucaacaaacggaa

SEQ ID NO: 2 - DNA, 21 bp, Artificial sequence
  DENV3_F3
cttaacgtagtgctgacagtt

SEQ ID NO: 3 - DNA, 18 bp, Artificial sequence
  DENV3_B3a
ctgctgttggtggaatgg

SEQ ID NO: 4 - DNA, 48 bp, Artificial sequence
  DENV3_FIPv4
tctcacgcgtttcagcatattgagagagcagatctctgatgaacaacc

SEQ ID NO: 5 - DNA, 42 bp, Artificial sequence
  DENV3_BIPv6
tggcgaagagattctcaagaggactagaaatctgaggaaagc

SEQ ID NO: 6 - DNA, 20 bp, Artificial sequence
  DENV3_LF
ttcccgtctttttccgttgg

SEQ ID NO: 7 - DNA, 17 bp, Artificial sequence
  DENV3_LBv1
attggttatggcgttta

SEQ ID NO: 8 - DNA, 30 bp, Artificial sequence
  DENV3_Qp
ctgaacggccaaggaccaatgaaattggtt

SEQ ID NO: 9 - DNA, 13 bp, Artificial sequence
  DENV3_B3-m12
atctagccaagac

SEQ ID NO: 10 - DNA, 13 bp, Artificial sequence
  DENV3_B3-m13
ctagccaagactc

SEQ ID NO: 11 - DNA, 13 bp, Artificial sequence
  DENV3_B3-m14
agccaagactcct

SEQ ID NO: 12 - DNA, 13 bp, Artificial sequence
  DENV3_B3-m16
gacttcttgaagg

SEQ ID NO: 13 - DNA, 13 bp, Artificial sequence
  DENV3_B3-m18
tcttgaaggttcc

SEQ ID NO: 14 - DNA, 13 bp, Artificial sequence
  DENV3_B3-m19
ttgaaggttcccc

SEQ ID NO: 15 - DNA, 13 bp, Artificial sequence
  DENV3_B3-m20
ttcttgaaggttc

SEQ ID NO: 16 - DNA, 13 bp, Artificial sequence
  DENV3_B3-m21
cttgaaggttccc

SEQ ID NO: 17 - DNA, 13 bp, Artificial sequence
  DENV3_B3-m23
aaggttccccatc

SEQ ID NO: 18 - DNA, 13 bp, Artificial sequence
  DENV3_B3-m25
ttgaaggttcccc

SEQ ID NO: 19 - DNA, 13 bp, Artificial sequence
  DENV3_B3-m26
gaaggttccccat

SEQ ID NO: 20 - DNA, 13 bp, Artificial sequence
  DENV3_B3-m27
aggttccccatct

SEQ ID NO: 21 - DNA, 13 bp, Artificial sequence
  DENV3_F4-1
gactcggaagctt

SEQ ID NO: 22 - DNA, 13 bp, Artificial sequence
  DENV3_F4-2
actcggaagcttg

SEQ ID NO: 23 - DNA, 14 bp, Artificial sequence
  DENV3_F4-3
gactcggaagcttg

SEQ ID NO: 24 - DNA, 12 bp, Artificial sequence
  DENV3_F4-4
gactcggaagct

SEQ ID NO: 25 - DNA, 12 bp, Artificial sequence
  DENV3_F4-5
actcggaagctt

SEQ ID NO: 26 - DNA, 12 bp, Artificial sequence
  DENV3_F4-6
ctcggaagcttg

SEQ ID NO: 27 - RNA, 1620 nt, Artificial sequence
  Hemagglutinin of Avian Influenza Virus (H5N1)
auggagaaaauagugcuucuuuuugcaauagucagucuuguuaaaagugaucagauuugcauugguuaccaugcaaacaacucgacagagcagguugacacaauaauggaaaagaacguuacuguuacacaugcccaagacauacuggaaaagaaacacaacgggaagcucugcgaucuagauggagugaagccucuaauuuugagagauuguagcguagcuggauggcuccucggaaacccaaugugugacgaauucaucaaugugccggaauggucuuacauaguggagaaggccaauccagucaaugaccucuguuacccaggggauuucaaugacuaugaagaauugaaacaccuauugagcagaauaaaccauuuugagaaaauucagaucauccccaaaaguucuugguccagucaugaagccucauuaggggugagcucagcauguccauaccagggaaaguccuccuuuuucagaaaugugguauggcuuaucaaaaagaacaguacauacccaacaauaaagaggagcuacaauaauaccaaccaagaagaucuuuugguacugugggggauucaccauccuaaugaugcggcagagcagacaaagcucuaucaaaacccaaccaccuauauuuccguugggacaucaacacuaaaccagagauugguaccaagaauagcuacuagauccaaaguaaacgggcaaaguggaaggauggaguucuucuggacaauuuuaaagccgaaugaugcaaucaacuucgagaguaauggaaauuucauugcuccagaauaugcauacaaaauugucaagaaaggggacucaacaauuaugaaaagugaauuggaauaugguaacugcaacaccaagugucaaacuccaaugggggcgauaaacucuagcaugccauuccacaauauacacccucucaccauuggggaaugccccaaauaugugaaaucaaacagauuaguccuugcgacugggcucagaaauagcccucaaagagagagaagaagaaaaaagagaggauuauuuggagcuauagcagguuuuauagagggaggauggcagggaaugguagaugguugguauggguaccaccauagcaaugagcaggggaguggguacgcugcagacaaagaauccacucaaaaggcaauagauggagucaccaauaaggucaacucgaucauugacaaaaugaacacucaguuugaggccguuggaagggaauuuaacaacuuagaaaggagaauagagaauuuaaacaagaagauggaagacggguuccuagaugucuggacuuauaaugcugaacuucugguucucauggaaaaugagagaacucuagacuuucaugacucaaaugucaagaaccuuuacgacaagguccgacuacagcuuagggauaaugcaaaggagcuggguaacgguuguuucgaguucuaucauaaaugugauaaugaauguauggaaaguguaagaaauggaacguaugacuacccgcaguauucagaagaagcgagacuaaaaagagaggaaauaaguggaguaaaauuggaaucaauaggaauuuaccaaauacugucaauuuauucuacaguggcg

SEQ ID NO: 28 - DNA, 19 bp, Artificial sequence
  H5N1-F3v7
caattttaaagccgaatga

SEQ ID NO: 29 - DNA, 17 bp, Artificial sequence
  H5N1-B3
gtcgcaaggactaatct

SEQ ID NO: 30 - DNA, 47 bp, Artificial sequence
  H5N1-FIP
accatattccaactcacttttcataatttcattgcaccagaatatgc

SEQ ID NO: 31 - DNA, 34 bp, Artificial sequence
  H5N1-BIP
caaactccaatgggggcatggtgagagggtgtat

SEQ ID NO: 32 - DNA, 20 bp, Artificial sequence
  H5N1-LF
gagtcccctttcttgacaat

SEQ ID NO: 33 - DNA, 19 bp, Artificial sequence
  H5N1-LB
gataaactctagtatgcca

SEQ ID NO: 34 - DNA, 12 bp, Artificial sequence
  H5N1-F4v2
aaagtggaagga

SEQ ID NO: 35 - DNA, 12 bp, Artificial sequence
  H5N1-F4v6
gggcaaagtgga

SEQ ID NO: 36 - DNA, 12 bp, Artificial sequence
  H5N1-F4v7
cgggcaaagtgg

SEQ ID NO: 37 - DNA, 13 bp, Artificial sequence
  H5N1-F4v17
gattggtaccaag

SEQ ID NO: 38 - DNA, 12 bp, Artificial sequence
  H5N1-B4v1
tttctgagccca

SEQ ID NO: 39 - DNA, 12 bp, Artificial sequence
  H5N1-B4v6
ggctatttctga

SEQ ID NO: 40 - DNA, 12 bp, Artificial sequence
  H5N1-B4v8
agggctatttct

SEQ ID NO: 41 - RNA, 1530 nt, Artificial sequence
  NS5 of ZIKV
guaauacgacucacuauagggaucaacaagguucguagcaaugcagcauuaggggcaauauuugaagaggaaaaagaguggaagacugcaguggaagcugugaacgauccaagguucugggcucuaguggacaaggaaagagagcaccaccugagaggagagugccagaguuguguguacaacaugaugggaaaaagagaaaagaaacaaggggaauuuggaaaggccaagggcagccgcgccaucugguauauguggcuaggggcuagauuucuagaguucgaagcccuuggauucuugaacgaggaucacuggauggggagagagaacucaggaggugguguugaagggcugggauuacaaagacucggauauguccuagaagagaugagucguauaccaggaggaaggauguaugcagaugacacugcuggcugggacacccgcauuagcagguuugaucuggagaaugaagcucuaaucaccaaccaaauggagaaagggcacagggccuuggcauuggccauaaucaaguacacauaccaaaacaaagugguaaagguccuuagaccagcugaaaaagggaaaacaguuauggacauuauuucgagacaagaccaaagggggagcggacaaguugucacuuacgcucuuaacacauuuaccaaccuaguggugcaacucauucggaauauggaggcugaggaaguucuagagaugcaagacuuguggcugcugcggaggucagagaaagugacuaacugguugcagagcaacggaugggauaggcucaaacgaauggcagucaguggagaugauugcguugugaagccaauugaugauagguuugcacaugcccucagguucuugaaugauaugggaaaaguuaggaaggacacacaagaguggaaacccucaacuggaugggacaacugggaagaaguuccguuuugcucccaccacuucaacaagcuccaucucaaggacgggagguccauugugguucccugccgccaccaagaugaacugauuggccgggcccgcgucucuccaggggcgggauggagcauccgggagacugcuugccuagcaaaaucauaugcgcaaauguggcagcuccuuuauuuccacagaagggaccuccgacugauggccaaugccauuuguucaucugugccaguugacuggguuccaacugggagaacuaccuggucaauccauggaaagggagaauggaugaccacugaagacaugcuugugguguggaacagaguguggauugaggagaacgaccacauggaagacaagaccccaguuacgaaauggacagacauucccuauuugggaaaaagggaagacuugugguguggaucucucauagggcacagaccgcgcaccaccugggcugagaacauuaaaaacacagucaacauggugcgcaggaucauaggugaugaagaaaaguacauggacuaccuauccacccaaguucgcuacuugggugaagaagggucuacaccuggagugcug

SEQ ID NO: 42 - DNA, 18 bp, Artificial sequence
  ZIKV F3
cagaagggacctccgact

SEQ ID NO: 43 - DNA, 20 bp, Artificial sequence
  ZIKV B3
cgtaactggggtcttgtctt

SEQ ID NO: 44 - DNA, 42 bp, Artificial sequence
  ZIKV FIP
ttgaccaggtagttctcccagtatggccaatgccatttgttc

SEQ ID NO: 45 - DNA, 42 bp, Artificial sequence
  ZIKV BIP
agggagaatggatgaccactgactcctcaatccacactctgt

SEQ ID NO: 46 - DNA, 18 bp, Artificial sequence
  ZIKV LF
cccagtcaactggcacag

SEQ ID NO: 47 - DNA, 15 bp, Artificial sequence
  ZIKV LB
catgcttgtggtgtg

SEQ ID NO: 48 - DNA, 29 bp, Artificial sequence
  ZIKV Qp
tggaacccagtcaactggcacagatgaac

SEQ ID NO: 49 - DNA, 14 bp, Artificial sequence
  ZIKV_B4-3
tagggaatgtctgt

SEQ ID NO: 50 - DNA, 12 bp, Artificial sequence
  ZIKV_B4-13
gaatgtctgtcc

SEQ ID NO: 51 - DNA, 13 bp, Artificial sequence
  ZIKV_B4-14
tgtctgtccattt

SEQ ID NO: 52 - DNA, 13 bp, Artificial sequence
  ZIKV_F4-2
ctcctttatttcc

SEQ ID NO: 53 - DNA, 17 bp, Artificial sequence
  ZIKV_F4-3
aaatcatatgcgcaaat

SEQ ID NO: 54 - RNA, 1374 nt, Artificial sequence
  N gene of RABV
auggaugccgacaagauuguguucaaagucaauaaucagguggucucuuugaagccugagauuaucguggaucaauaugaguacaaguacccugccaucaaggauuugaaaaagccuuguaucacccuagggaaagcccccgacuugaacaaagcauacaaaucaguuuuaucaggcaugaaugccgccaaacuugauccggaugauguaugcuccuacuuggcagcagcaaugcaguucuuugaggggacauguccggaagacuggaccagcuauggaauccugauugcacgaaaaggagacaggaucaccccaaacucucuaguggagauaaagcguacugauguagacgggaauugggcucugacaggaggcauggaauugacaagggaccccacugucucugaacaugcaucuuuagucggucuucuccugagucuguacagguugagcaaaauaucaggacagaacacugguaacuauaagacaaacauugcagauaggauagagcagauuuucgagacagcaccuuuuguuaagaucguggaacaccauacccuaaugacaacucacaagaugugugcuaauuggaguacuauaccgaacuucagauuuuuggccggaaccuacgacauguuuuucucacggauugagcaucuguauucggcaaucagagugggcacagucgucaccgcuuaugaagacugcucaggacugguaucguuuacaggguucauaaagcagaucaaucucaccgcaagggaagcaauacuauauuucuuccacaagaacuuugaggaagagauaagaagaauguucgagccagggcaagagacagcuguuccucacucuuauuucauccacuuccguucacuaggcuugagugggaagucuccuuauucaucgaaugcugucggucauguguucaaucucauucacuuuguuggaugcuacaugggucaagucagaucucuaaaugcgacgguuauugcugcaugugccccucaugagaugucuguucuagggggcuauuugggagaggaauucuucggaaaagggacauuugaaagaagguucuucagagacgagaaagaacuucaagaauaugaggcggcugaacuaacaaagaccgacguggcacuggcagaugacggaaccgucaacucugaugacgaggacuauuucuccggugaaaccagaaguccagaagcugucuauacucgaaucaugaugaauggaggucgacugaagagaucucauauacggagauaugucucagucaguuccaaucaucaagcccguccaaacucauucgccgaauuuuuaaacaagacguauucgaaugacucauaacccuauagugagucguauuac

SEQ ID NO: 55 - DNA, 16 bp, Artificial sequence
  RABV1-F3
acatgtccggaagact

SEQ ID NO: 56 - DNA, 18 bp, Artificial sequence
  RABV1-B3
cagactcaggagaagacc

SEQ ID NO: 57 - DNA, 37 bp, Artificial sequence
  RABV1-FIP
actagagagtttggggtgaggaccagctatggaatcc

SEQ ID NO: 58 - DNA, 37 bp, Artificial sequence
  RABV1-BIP
acgggaattgggctctgacctaaagatgcatgttcag

SEQ ID NO: 59 - DNA, 22 bp, Artificial sequence
  RABV1-LB
ggcatggaattgacaagggacc

SEQ ID NO: 60 - DNA, 13 bp, Artificial sequence
  RABV1-F4v14
cagcagcaatgca

SEQ ID NO: 61 - DNA, 14 bp, Artificial sequence
  RABV1-B4v3
tattttgctcaacc

SEQ ID NO: 62 - DNA, 14 bp, Artificial sequence
  RABV1-B4v7
tgtcctgatatttt